European Patent Specification EP 3 399 045 B9, published October 4, 2023. Title: Heparan sulfate having high 3-O-sufation rate of glucosamine residue. Applicant: Ajinomoto Co., Inc. The sequence listing filed with the application follows.

SEQUENCE LISTING (41 sequences)

SEQ ID NO: 1 - DNA, 7467 bp, Escherichia coli
  CDS (445)..(1164)
  CDS (1593)..(3284)
  CDS (4576)..(6138)
  CDS (6180)..(7358)
ggaggcctgattactgttgcactaacagtgtcattgccggagattgtaatcacactctatataattatataaactctattgtatttagtgtatgaggaggatggacagtatactttgaactaggtaattatgaatttgatcgtgatctcgtaatacgttgctgttattctttaattaattatctgccaatttatttttagatagttacaggaaatgtttatgcaaagagtggtttgatatggtaagagtaataatttagatgaagataaatatatcaaacgtacaccctagtagttatttttaattaaacatatcgtccatgaggtgcggagtcattctaatcaacttaatgtgttctgtttattaagcatttcctataaataaacgactatcaatacgttgatagttttcattaacatgcaatattaattaaaatattaccccatgattgttgcaaatatgtcatcatacccacctcgaaaaaaagagttggtgcattctatacaaagtttacatgctcaagtagataaaattaatctttgcctgaatgagtttgaagaaattcctgaggaattagatggtttttcaaaattaaatccagttattccagataaagattataaggatgtgggcaaatttatatttccttgcgctaaaaatgatatgatcgtacttacagatgatgatattatttaccctcccgattatgtagaaaaaatgctcaatttttataattcctttgcaatattcaattgcattgttgggattcatggctgtatatacatagatgcatttgatggagatcagtctaaaagaaaagtattttcatttactcaagggctattgcgaccgagagttgtaaatcaattaggtacagggactgtttttcttaaggcagatcaattaccatctttaaaatatatggatggttctcaacgattcgtcgatgttagattttctcgctatatgttagagaatgaaattggtatgatatgtgttcccagagaaaaaaactggctaagagaggtctcatcaggttcaatggaaggactttggaacacatttacaaaaaaatggcctttagacatcataaaagaaacacaagcaatcgcaggatattcaaaacttaacctcgaattagtgtataatgtggaagggtaaaaacttacttttttattcacattcctgtattttgtgttggtttctgaagtttatagtataaatacttgttttaaatagttgtacgttgatattttgttatatacttatttaaaccatttgttttatgattttgaaaaatatcagcgttagtttggtagagtttataattaagatttttgtctaaaagaaggtggtaacgcaatatgtcaattattaggaggtgctctgagttatattgatattgtttattgatgaatggctataccaaataaatcagatgtgctattgagatatagatagtttcatttagtattatcacataacgccacctaaattacattacagatttgaaatatatgtctgcaatatcaccattacgataaacgacagtgtttaaaataaagtaatcttgtagataataaagaggaaatatgatgaataaattagtgctagtcggacatcctggctcaaagtatcagatagttgaacattttttgaaagaaattggcatgaactcaccaaattattctacaagtaataaaatttccccagaatatatcaccgcttcattatgtcaattttatcaaacaccagaagttaatgatgtagtagatgagagagaattctcagctgttcaagtctcaaccatgtgggatagcatggttcttgaactaatgatgaacaatctaaataacaaactttgggggtgggcagatccatctataatattttttcttgatttttggaaaaatatagataaaagcataaaattcatcatgatatatgatcaccctaaatataatttaatgcgttcagtaaataatgcccctctctctttaaatataaataatagtgtagataactggattgcatataataaaagattgcttgatttttttttggagaataaagaacgatgtgtgttgattaattttgaggcgtttcaaagcaataagaaaaatattataaagccattgagtaatattataaaaatagataatctaatgtctgcgcattacaaaaattcaatattgtttgatgtggttgagaataatgattatacaaaatcaaatgaaattgccctgcttgaaaaatatacaactttattttctttaagtgcaaatgagactgaaattacatttaatgatacaaaggttagtgagtacttagtatctgaattaataaaagaaagaaccgaggttctgaagctttataatgagttacaagcctatgcaaacctaccttatatagaaacatcgaaagataacgtttcggctgaggctgcattatgggaggtagtcgaagagagaaattctatcttcaatattgtatctcatttggtgcaagagtcaaaaaagaaggatgcagatattgaattgactaaatctatatttaagaaaagacaatttttattattgaacaggattaatgagctaaaaaaagaaaaggaagaggtaattaaactttcaaaaataaatcacaacgatgttgtgagacaagaaaaatatccagatgatattgaaaaaaaaataaatgacatacagaaatatgaagaagagataagcgaaaaagaatcaaaactcactcaggcaatatcagaaaaagaacagattttaaaacaattgcataaatatgaagaagagataagcgaaaaagaatcaaaactcactcaggcaatatcagaaaaagaacagattttaaaacaattgcatatagtgcaagagcagttggaacactattttatagaaaatcaggaaattaaaaagaaacttccacctgtgctatatggagcagctgagcagataaaacaagagttaggttatcgacttggttatattatagtctcgtattctaaatccctcaaggggattattaccatgccatttgcacttatccgtgagtgtgtttttgaaaaaaaacgtaagaagagttatggcgttgatgtgccactctatttatatgctgatgctgataaggctgaaagagttaagaaacatttatcttatcaattagggcaggctattatctccagtgctaattcgatatttggattcattacccttccatttaagttaattgttgttgtttataaatataggagagctaaaatcaagggctgttaaaaatgtgaaccctaatgagatatattgcaaattttatttttctctttgtggtgttttgctttcgttaaaatagttagttattttatttatataatatcacgcattataataccaatttatacttttgcaagtgaccgtatagattcgccacatattgcaaattttgttctctcgtaaaatattttcttctggtgtcagtaattcgagcacttcatgctgtcttttactgcagtatagtactaggttttcagctagtttctgattaaatatgtttagctctttaaagagtctatttatttaaattcaatgaactgttctttcggcgttcgcttaaaacgttcagaggtgcgttctaggcgtaaaggggtaggtccatagggcttgctagcggattcctgcggtgctttgtcgaagtttcctgggaactctttcccgttatctgcgatgccctggttgatatcgatagggaatagccggtctgcacggcaaaagaagagtttgatgatatcacagttaagtgacggcacggcctgtgccagagcgtagttgctgtgttcgtcgatcatggtaatgacataacagcgcagctcgcccattctgagctcaatagcatctataccaacgagctcactgctctttaccgggcgatagcgttttgatctgcgggttggaggattgtattttttatgaacagtgtttttccttggggaggcagtcacatcggtatcagtcgcattttatcgtgtgcggccgtgaacatcctgccgatggttgaaatgctcggacagaccaggcggtgctgttcactccacggcttcaagcaaacaaaaatctgttcttctaggttgggaagctctattctcagtcgacgtatttcttacagaattacgagatgccattgctttgtgcgatgtactagcggagctttgctacgcgaaataggtgcctctgggccataatacagcgttcgtgtggatacagcaaaaacttccgcaactgtattgatctcatgtttctcccagaagtatattttttcatccttaattttgtaatctcaggtataacaaagtgtttcatcacatagatgttggcatggtaatgcctcaaatatccgccgcagatacgttgcatcaacttagcatttccctcgcttgtccggagataattgcaatatctctgtgagcttacactgtgacattcgttgagttttagtgatgtttttaaagatttatatttataatatttagtaaatgcagttttattctcattttatttatcattaagtgaatgtatgaacgcagaatatataaatttagttgaacgtaaaaagaaattagggacaaatattggtgctcttgattttttattatcaattcataaggagaaagttgatcttcaacataaaaactcgcctttaaaaggtaacgataaccttattcacaaaagaataaacgaatacgacaatgtacttgaactatctaagaatgtatcagctcagaattctggcaatgagttttcttatttattgggatatgcagattctcttagaaaagttggtatgttggatacttatattaaaattgtttgttatctaacaattcaatctcgttattttaaaaatggcgaacgagttaagctttttgaacatataagtaacgctctacggtattcaaggagtgattttctcattaatcttatttttgaacgatatatcgaatatataaaccatctaaaattgtcgcccaaacaaaaagatttttatttttgtacgaagttttcaaaatttcatgattatactaaaaatggatataaatatttagcatttgataatcaagccgatgcagggtatggcctgactttattattaaatgcaaacgatgatatgcaagatagttataatctactccctgagcaagaactttttatttgtaatgctgtaatagataatatgaatatttataggagtcaatttaacaaatgtctacgaaaatacgatttatcagaaataactgatatatacccaaataaaattatattgcaaggaattaagttcgataagaaaaaaaatgtttatggaaaagatcttgttagtataataatgtcagtattcaattcagaagatactattgcatactcattacattcattgttgaatcaaacatatgaaaatattgaaattctcgtgtgcgatgattgttcatcggacaaaagccttgaaataattaagagcatagcttattctgattcaagagtgaaagtatatagctcacgaaaaaaccaaggcccttataatataagaaatgagctaataaaaaaagcacacggtaatttcatcacctttcaagatgcagatgatctttctcatccggagagaatacaaagacaagttgaggttcttcgcaataataaggctgtaatctgtatggctaactggatccgtgttgcgtcaaatggaaaaattcaattcttctatgatgataaagccacaagaatgtctgttgtatcgtcaatgataaaaaaagatatttttgcgacagttggtggctatagacaatctttaattggtgcagatacggagttttatgaaacagtaataatgcgttatgggcgagaaagtattgtaagattactgcagccattgatattggggttatggggagactccggacttaccaggaataaaggaacagaagctctacctgatggatatatatcacaatctcgaagagaatatagtgatatcgcggcaagacaacgagtgttagggaaaagtatcgtaagtgataaagatgtacgtggtttattatctcgctatggtttgtttaaagatgtatcaggaataattgaacaatagtttgttattctatatatattaaatttttggggctatataaaatgttcggaacactaaaaataactgtttcaggcgctggttacgttgggctttcaaatggaattctaatggctcaaaatcatgaagtggttgcatttgatacccatcaaaaaaaagttgacttacttaatgataaactctctcctatagaggataaggaaattgaaaattatctttcaactaaaatacttaattttcgcgcaactactaacaaatatgaagcctataaaaatgccaattacgttattattgctacaccaacgaattatgacccaggttcaaattactttgatacatcaagcgttgaagctgtcattcgtgacgtaacggaaatcaacccaaacgcaattatggtggttaaatctacggtcccagtaggtttcacaaaaacaattaaagaacatttaggtattaataatattatcttctctccagaatttttacgagaaggaagagccctatacgataatctccatccatctcgcattattatcggtgaatgttctgaacgggcagaacgtttggcagtgttatttcaggaaggagcgattaaacaaaatatacccgttttatttacagattctacggaagcggaagcgattaagttattttcaaatacttatttggctatgcgagttgcattttttaatgaattggatagttacgcagaaagttttggtctgaatacgcgtcagattattgacggtgtttgtttggatccgcgcattggtaattactacaataatccttcttttggttatggtggctactgtttgccaaaagataccaagcaattattagccaactatcagtctgttccgaataaacttatatctgcaattgttgatgctaaccgtacacgtaaggactttatcactaatgttattttgaaacatagaccacaagttgtgggggtttatcgtttgattatgaaaagtggttcagataattttagagattcttctattcttggtattataaagcgtatcaagaaaaaaggcgtgaaagtaattatttatgagccgcttatttctggagatacattctttaactcacctttggaacgggagctggcgatctttaaagggaaagctgatattattatcactaaccgaatgtcagaggagttgaacgatgtggtcgacaaagtctatagtcgcgatttgtttaaatgtgactaatgtattgttatatactattaactattaagagaaggaaatgcattatttaatccgttaaaaatatgcctcgttggtatgttctttattaatcctcgatcgtaaaataaga

SEQ ID NO: 2 - protein, 238 aa, Escherichia coli
MIVANMSSYPPRKKELVHSIQSLHAQVDKINLCLNEFEEIPEELDGFSKLNPVIPDKDYKDVGKFIFPCAKNDMIVLTDDDIIYPPDYVEKMLNFYNSFAIFNCIVGIHGCIYIDAFDGDQSKRKVFSFTQGLLRPRVVNQLGTGTVFLKADQLPSLKYMDGSQRFVDVRFSRYMLENEIGMICVPREKNWLREVSSGSMEGLWNTFTKKWPLDIIKETQAIAGYSKLNLELVYNVEG

SEQ ID NO: 3 - protein, 563 aa, Escherichia coli
MMNKLVLVGHPGSKYQIVEHFLKEIGMNSPNYSTSNKISPEYITASLCQFYQTPEVNDVVDEREFSAVQVSTMWDSMVLELMMNNLNNKLWGWADPSIIFFLDFWKNIDKSIKFIMIYDHPKYNLMRSVNNAPLSLNINNSVDNWIAYNKRLLDFFLENKERCVLINFEAFQSNKKNIIKPLSNIIKIDNLMSAHYKNSILFDVVENNDYTKSNEIALLEKYTTLFSLSANETEITFNDTKVSEYLVSELIKERTEVLKLYNELQAYANLPYIETSKDNVSAEAALWEVVEERNSIFNIVSHLVQESKKKDADIELTKSIFKKRQFLLLNRINELKKEKEEVIKLSKINHNDVVRQEKYPDDIEKKINDIQKYEEEISEKESKLTQAISEKEQILKQLHKYEEEISEKESKLTQAISEKEQILKQLHIVQEQLEHYFIENQEIKKKLPPVLYGAAEQIKQELGYRLGYIIVSYSKSLKGIITMPFALIRECVFEKKRKKSYGVDVPLYLYADADKAERVKKHLSYQLGQAIISSANSIFGFITLPFKLIVVVYKYRRAKIKGC

SEQ ID NO: 4 - protein, 520 aa, Escherichia coli
MNAEYINLVERKKKLGTNIGALDFLLSIHKEKVDLQHKNSPLKGNDNLIHKRINEYDNVLELSKNVSAQNSGNEFSYLLGYADSLRKVGMLDTYIKIVCYLTIQSRYFKNGERVKLFEHISNALRYSRSDFLINLIFERYIEYINHLKLSPKQKDFYFCTKFSKFHDYTKNGYKYLAFDNQADAGYGLTLLLNANDDMQDSYNLLPEQELFICNAVIDNMNIYRSQFNKCLRKYDLSEITDIYPNKIILQGIKFDKKKNVYGKDLVSIIMSVFNSEDTIAYSLHSLLNQTYENIEILVCDDCSSDKSLEIIKSIAYSDSRVKVYSSRKNQGPYNIRNELIKKAHGNFITFQDADDLSHPERIQRQVEVLRNNKAVICMANWIRVASNGKIQFFYDDKATRMSVVSSMIKKDIFATVGGYRQSLIGADTEFYETVIMRYGRESIVRLLQPLILGLWGDSGLTRNKGTEALPDGYISQSRREYSDIAARQRVLGKSIVSDKDVRGLLSRYGLFKDVSGIIEQ

SEQ ID NO: 5 - protein, 392 aa, Escherichia coli
MFGTLKITVSGAGYVGLSNGILMAQNHEVVAFDTHQKKVDLLNDKLSPIEDKEIENYLSTKILNFRATTNKYEAYKNANYVIIATPTNYDPGSNYFDTSSVEAVIRDVTEINPNAIMVVKSTVPVGFTKTIKEHLGINNIIFSPEFLREGRALYDNLHPSRIIIGECSERAERLAVLFQEGAIKQNIPVLFTDSTEAEAIKLFSNTYLAMRVAFFNELDSYAESFGLNTRQIIDGVCLDPRIGNYYNNPSFGYGGYCLPKDTKQLLANYQSVPNKLISAIVDANRTRKDFITNVILKHRPQVVGVYRLIMKSGSDNFRDSSILGIIKRIKKKGVKVIIYEPLISGDTFFNSPLERELAIFKGKADIIITNRMSEELNDVVDKVYSRDLFKCD

SEQ ID NO: 6 - DNA, 36 bp, Artificial Sequence
  primer
agctgagtcgacccccaggaaaaattggttaataac

SEQ ID NO: 7 - DNA, 33 bp, Artificial Sequence
  primer
agctgagcatgcttccaactgcgctaatgacgc

SEQ ID NO: 8 - DNA, 313 bp, Artificial Sequence
  promoter
gcatgcttccaactgcgctaatgacgcagctggacgaaggcgggattctcgtcttacccgtaggggaggagcaccagtatttgaaacgggtgcgtcgtcggggaggcgaatttattatcgataccgtggaggccgtgcgctttgtccctttagtgaagggtgagctggcttaaaacgtgaggaaatacctggatttttcctggttattttgccgcaggtcagcgtatcgtgaacatcttttccagtgttcagtagggtgccttgcacggtaattatgtcactggttattaaccaatttttcctgggggtcgac

SEQ ID NO: 9 - DNA, 33 bp, Artificial Sequence
  primer
agctgatctagaaaacagaatttgcctggcggc

SEQ ID NO: 10 - DNA, 33 bp, Artificial Sequence
  primer
agctgaggatccaggaagagtttgtagaaacgc

SEQ ID NO: 11 - DNA, 369 bp, Artificial Sequence
  terminator
tctagaaacagaatttgcctggcggcagtagcgcggtggtcccacctgaccccatgccgaactcagaagtgaaacgccgtagcgccgatggtagtgtggggtctccccatgcgagagtagggaactgccaggcatcaaataaaacgaaaggctcagtcgaaagactgggcctttcgttttatctgttgtttgtcggtgaacgctctcctgagtaggacaaatccgccgggagcggatttgaacgttgcgaagcaacggcccggagggtggcgggcaggacgcccgccataaactgccaggcatcaaattaagcagaaggccatcctgacggatggcctttttgcgtttctacaaactcttcctggatcc

SEQ ID NO: 12 - DNA, 35 bp, Artificial Sequence
  primer
ttcctgggggtcgacatgactacgaaaatttttaa

SEQ ID NO: 13 - DNA, 35 bp, Artificial Sequence
  primer
attctgttttctagactaaggaaccaacacaagct

SEQ ID NO: 14 - DNA, 30 bp, Artificial Sequence
  primer
gtcgacccccaggaaaaattggttaataac

SEQ ID NO: 15 - DNA, 30 bp, Artificial Sequence
  primer
tctagaaaacagaatttgcctggcggcagt

SEQ ID NO: 16 - DNA, 1980 bp, Flavobacterium heparinum
atgactacgaaaatttttaaaaggatcattgtatttgctgtaattgccctatcgtcgggaaatatacttgcacaaagctcttccattaccaggaaagattttgaccacatcaaccttgagtattccggactggaaaaggttaataaagcagttgctgccggcaactatgacgatgcggccaaagcattactggcatactacagggaaaaaagtaaggccagggaacctgatttcagtaatgcagaaaagcctgccgatatacgccagcccatagataaggttacgcgtgaaatggccgacaaggctttggtccaccagtttcaaccgcacaaaggctacggctattttgattatggtaaagacatcaactggcagatgtggccggtaaaagacaatgaagtacgctggcagttgcaccgtgtaaaatggtggcaggctatggccctggtttatcacgctacgggcgatgaaaaatatgcaagagaatgggtatatcagtacagcgattgggccagaaaaaacccattgggcctgtcgcaggataatgataaatttgtgtggcggccccttgaagtgtcggacagggtacaaagtcttcccccaaccttcagcttatttgtaaactcgccagcctttaccccagcctttttaatggaatttttaaacagttaccaccaacaggccgattatttatctacgcattatgccgaacagggaaaccaccgtttatttgaagcccaacgcaacttgtttgcaggggtatctttccctgaatttaaagattcaccaagatggaggcaaaccggcatatcggtgctgaacaccgagatcaaaaaacaggtttatgccgatgggatgcagtttgaactttcaccaatttaccatgtagctgccatcgatatcttcttaaaggcctatggttctgcaaaacgagttaaccttgaaaaagaatttccgcaatcttatgtacaaactgtagaaaatatgattatggcgctgatcagtatttcactgccagattataacacccctatgtttggagattcatggattacagataaaaatttcaggatggcacagtttgccagctgggcccgggttttcccggcaaaccaggccataaaatattttgctacagatggcaaacaaggtaaggcgcctaactttttatccaaagcattgagcaatgcaggcttttatacgtttagaagcggatgggataaaaatgcaaccgttatggtattaaaagccagtcctcccggagaatttcatgcccagccggataacgggacttttgaactttttataaagggcagaaactttaccccagacgccggggtatttgtgtatagcggcgacgaagccatcatgaaactgcggaactggtaccgtcaaacccgcatacacagcacgcttacactcgacaatcaaaatatggtcattaccaaagcccggcaaaacaaatgggaaacaggaaataaccttgatgtgcttacctataccaacccaagctatccgaatctggaccatcagcgcagtgtacttttcatcaacaaaaaatactttctggtcatcgatagggcaataggcgaagctaccggaaacctgggcgtacactggcagcttaaagaagacagcaaccctgttttcgataagacaaagaaccgggtttacaccacttacagagatggtaacaacctgatgatccaatcgttgaatgcggacaggaccagcctcaatgaagaagaaggaaaggtatcttatgtttacaataaggagctgaaaagacctgctttcgtatttgaaaagcctaaaaagaatgccggcacacaaaattttgtcagtatagtttatccatacgacggccagaaggctccagagatcagcatacgggaaaacaagggcaatgattttgagaaaggcaagcttaatctaacccttaccattaacggaaaacaacagcttgtgttggttccttag

SEQ ID NO: 17 - protein, 659 aa, Flavobacterium heparinum
MTTKIFKRIIVFAVIALSSGNILAQSSSITRKDFDHINLEYSGLEKVNKAVAAGNYDDAAKALLAYYREKSKAREPDFSNAEKPADIRQPIDKVTREMADKALVHQFQPHKGYGYFDYGKDINWQMWPVKDNEVRWQLHRVKWWQAMALVYHATGDEKYAREWVYQYSDWARKNPLGLSQDNDKFVWRPLEVSDRVQSLPPTFSLFVNSPAFTPAFLMEFLNSYHQQADYLSTHYAEQGNHRLFEAQRNLFAGVSFPEFKDSPRWRQTGISVLNTEIKKQVYADGMQFELSPIYHVAAIDIFLKAYGSAKRVNLEKEFPQSYVQTVENMIMALISISLPDYNTPMFGDSWITDKNFRMAQFASWARVFPANQAIKYFATDGKQGKAPNFLSKALSNAGFYTFRSGWDKNATVMVLKASPPGEFHAQPDNGTFELFIKGRNFTPDAGVFVYSGDEAIMKLRNWYRQTRIHSTLTLDNQNMVITKARQNKWETGNNLDVLTYTNPSYPNLDHQRSVLFINKKYFLVIDRAIGEATGNLGVHWQLKEDSNPVFDKTKNRVYTTYRDGNNLMIQSLNADRTSLNEEEGKVSYVYNKELKRPAFVFEKPKKNAGTQNFVSIVYPYDGQKAPEISIRENKGNDFEKGKLNLTLTINGKQQLVLVP

SEQ ID NO: 18 - DNA, 44 bp, Artificial Sequence
  primer
ttcagaattcggatccaataaatgtagcagcgataaagcaattc

SEQ ID NO: 19 - DNA, 44 bp, Artificial Sequence
  primer
ggccagtgccaagcttttaattgtgttttgcacggctacctttc

SEQ ID NO: 20 - DNA, 6646 bp, Artificial Sequence
  plasmid
ccgacaccatcgaatggtgcaaaacctttcgcggtatggcatgatagcgcccggaagagagtcaattcagggtggtgaatgtgaaaccagtaacgttatacgatgtcgcagagtatgccggtgtctcttatcagaccgtttcccgcgtggtgaaccaggccagccacgtttctgcgaaaacgcgggaaaaagtggaagcggcgatggcggagctgaattacattcccaaccgcgtggcacaacaactggcgggcaaacagtcgttgctgattggcgttgccacctccagtctggccctgcacgcgccgtcgcaaattgtcgcggcgattaaatctcgcgccgatcaactgggtgccagcgtggtggtgtcgatggtagaacgaagcggcgtcgaagcctgtaaagcggcggtgcacaatcttctcgcgcaacgcgtcagtgggctgatcattaactatccgctggatgaccaggatgccattgctgtggaagctgcctgcactaatgttccggcgttatttcttgatgtctctgaccagacacccatcaacagtattattttctcccatgaagacggtacgcgactgggcgtggagcatctggtcgcattgggtcaccagcaaatcgcgctgttagcgggcccattaagttctgtctcggcgcgtctgcgtctggctggctggcataaatatctcactcgcaatcaaattcagccgatagcggaacgggaaggcgactggagtgccatgtccggttttcaacaaaccatgcaaatgctgaatgagggcatcgttcccactgcgatgctggttgccaacgatcagatggcgctgggcgcaatgcgcgccattaccgagtccgggctgcgcgttggtgcggatatctcggtagtgggatacgacgataccgaagacagctcatgttatatcccgccgttaaccaccatcaaacaggattttcgcctgctggggcaaaccagcgtggaccgcttgctgcaactctctcagggccaggcggtgaagggcaatcagctgttgcccgtctcactggtgaaaagaaaaaccaccctggcgcccaatacgcaaaccgcctctccccgcgcgttggccgattcattaatgcagctggcacgacaggtttcccgactggaaagcgggcagtgagcgcaacgcaattaatgtaagttagctcactcattaggcacaattctcatgtttgacagcttatcatcgactgcacggtgcaccaatgcttctggcgtcaggcagccatcggaagctgtggtatggctgtgcaggtcgtaaatcactgcataattcgtgtcgctcaaggcgcactcccgttctggataatgttttttgcgccgacatcataacggttctggcaaatattctgaaatgagctgttgacaattaatcatcggctcgtataatgtgtggaattgtgagcggataacaatttcacacaggaaacagccagtccgtttaggtgttttcacgagcacttcaccaacaaggaccatagcatatgaaaatcgaagaaggtaaactggtaatctggattaacggcgataaaggctataacggtctcgctgaagtcggtaagaaattcgagaaagataccggaattaaagtcaccgttgagcatccggataaactggaagagaaattcccacaggttgcggcaactggcgatggccctgacattatcttctgggcacacgaccgctttggtggctacgctcaatctggcctgttggctgaaatcaccccggacaaagcgttccaggacaagctgtatccgtttacctgggatgccgtacgttacaacggcaagctgattgcttacccgatcgctgttgaagcgttatcgctgatttataacaaagatctgctgccgaacccgccaaaaacctgggaagagatcccggcgctggataaagaactgaaagcgaaaggtaagagcgcgctgatgttcaacctgcaagaaccgtacttcacctggccgctgattgctgctgacgggggttatgcgttcaagtatgaaaacggcaagtacgacattaaagacgtgggcgtggataacgctggcgcgaaagcgggtctgaccttcctggttgacctgattaaaaacaaacacatgaatgcagacaccgattactccatcgcagaagctgcctttaataaaggcgaaacagcgatgaccatcaacggcccgtgggcatggtccaacatcgacaccagcaaagtgaattatggtgtaacggtactgccgaccttcaagggtcaaccatccaaaccgttcgttggcgtgctgagcgcaggtattaacgccgccagtccgaacaaagagctggcaaaagagttcctcgaaaactatctgctgactgatgaaggtctggaagcggttaataaagacaaaccgctgggtgccgtagcgctgaagtcttacgaggaagagttggcgaaagatccacgtattgccgccactatggaaaacgcccagaaaggtgaaatcatgccgaacatcccgcagatgtccgctttctggtatgccgtgcgtactgcggtgatcaacgccgccagcggtcgtcagactgtcgatgaagccctgaaagacgcgcagactaattcgagctcgaacaacaacaacaataacaataacaacaacctcgggatcgagggaaggatttcagaattcggatcctctagagtcgacctgcaggcaagcttggcactggccgtcgttttacaacgtcgtgactgggaaaaccctggcgttacccaacttaatcgccttgcagcacatccccctttcgccagctggcgtaatagcgaagaggcccgcaccgatcgcccttcccaacagttgcgcagcctgaatggcgaatggcagcttggctgttttggcggatgagataagattttcagcctgatacagattaaatcagaacgcagaagcggtctgataaaacagaatttgcctggcggcagtagcgcggtggtcccacctgaccccatgccgaactcagaagtgaaacgccgtagcgccgatggtagtgtggggtctccccatgcgagagtagggaactgccaggcatcaaataaaacgaaaggctcagtcgaaagactgggcctttcgttttatctgttgtttgtcggtgaacgctctcctgagtaggacaaatccgccgggagcggatttgaacgttgcgaagcaacggcccggagggtggcgggcaggacgcccgccataaactgccaggcatcaaattaagcagaaggccatcctgacggatggcctttttgcgtttctacaaactctttttgtttatttttctaaatacattcaaatatgtatccgctcatgagacaataaccctgataaatgcttcaataatattgaaaaaggaagagtatgagtattcaacatttccgtgtcgcccttattcccttttttgcggcattttgccttcctgtttttgctcacccagaaacgctggtgaaagtaaaagatgctgaagatcagttgggtgcacgagtgggttacatcgaactggatctcaacagcggtaagatccttgagagttttcgccccgaagaacgttctccaatgatgagcacttttaaagttctgctatgtggcgcggtattatcccgtgttgacgccgggcaagagcaactcggtcgccgcatacactattctcagaatgacttggttgagtactcaccagtcacagaaaagcatcttacggatggcatgacagtaagagaattatgcagtgctgccataaccatgagtgataacactgcggccaacttacttctgacaacgatcggaggaccgaaggagctaaccgcttttttgcacaacatgggggatcatgtaactcgccttgatcgttgggaaccggagctgaatgaagccataccaaacgacgagcgtgacaccacgatgcctgtagcaatggcaacaacgttgcgcaaactattaactggcgaactacttactctagcttcccggcaacaattaatagactggatggaggcggataaagttgcaggaccacttctgcgctcggcccttccggctggctggtttattgctgataaatctggagccggtgagcgtgggtctcgcggtatcattgcagcactggggccagatggtaagccctcccgtatcgtagttatctacacgacggggagtcaggcaactatggatgaacgaaatagacagatcgctgagataggtgcctcactgattaagcattggtaactgtcagaccaagtttactcatatatactttagattgatttaccccggttgataatcagaaaagccccaaaaacaggaagattgtataagcaaatatttaaattgtaaacgttaatattttgttaaaattcgcgttaaatttttgttaaatcagctcattttttaaccaataggccgaaatcggcaaaatcccttataaatcaaaagaatagaccgagatagggttgagtgttgttccagtttggaacaagagtccactattaaagaacgtggactccaacgtcaaagggcgaaaaaccgtctatcagggcgatggcccactacgtgaaccatcacccaaatcaagttttttggggtcgaggtgccgtaaagcactaaatcggaaccctaaagggagcccccgatttagagcttgacggggaaagccggcgaacgtggcgagaaaggaagggaagaaagcgaaaggagcgggcgctagggcgctggcaagtgtagcggtcacgctgcgcgtaaccaccacacccgccgcgcttaatgcgccgctacagggcgcgtaaaaggatctaggtgaagatcctttttgataatctcatgaccaaaatcccttaacgtgagttttcgttccactgagcgtcagaccccgtagaaaagatcaaaggatcttcttgagatcctttttttctgcgcgtaatctgctgcttgcaaacaaaaaaaccaccgctaccagcggtggtttgtttgccggatcaagagctaccaactctttttccgaaggtaactggcttcagcagagcgcagataccaaatactgtccttctagtgtagccgtagttaggccaccacttcaagaactctgtagcaccgcctacatacctcgctctgctaatcctgttaccagtggctgctgccagtggcgataagtcgtgtcttaccgggttggactcaagacgatagttaccggataaggcgcagcggtcgggctgaacggggggttcgtgcacacagcccagcttggagcgaacgacctacaccgaactgagatacctacagcgtgagctatgagaaagcgccacgcttcccgaagggagaaaggcggacaggtatccggtaagcggcagggtcggaacaggagagcgcacgagggagcttccagggggaaacgcctggtatctttatagtcctgtcgggtttcgccacctctgacttgagcgtcgatttttgtgatgctcgtcaggggggcggagcctatggaaaaacgccagcaacgcggcctttttacggttcctggccttttgctggccttttgctcacatgttctttcctgcgttatcccctgattctgtggataaccgtattaccgcctttgagtgagctgataccgctcgccgcagccgaacgaccgagcgcagcgagtcagtgagcgaggaagcggaagagcgcctgatgcggtattttctccttacgcatctgtgcggtatttcacaccgcatatatggtgcactctcagtacaatctgctctgatgccgcatagttaagccagtatacactccgctatcgctacgtgactgggtcatggctgcgccccgacacccgccaacacccgctgacgcgccctgacgggcttgtctgctcccggcatccgcttacagacaagctgtgaccgtctccgggagctgcatgtgtcagaggttttcaccgtcatcaccgaaacgcgcgaggcagctgcggtaaagctcatcagcgtggtcgtgcagcgattcacagatgtctgcctgttcatccgcgtccagctcgttgagtttctccagaagcgttaatgtctggcttctgataaagcgggccatgttaagggcggttttttcctgtttggtcactgatgcctccgtgtaagggggatttctgttcatgggggtaatgataccgatgaaacgagagaggatgctcacgatacgggttactgatgatgaacatgcccggttactggaacgttgtgagggtaaacaactggcggtatggatgcggcgggaccagagaaaaatcactcagggtcaatgccagcgcttcgttaatacagatgtaggtgttccacagggtagccagcagcatcctgcgatgcagatccggaacataatggtgcagggcgctgacttccgcgtttccagactttacgaaacacggaaaccgaagaccattcatgttgttgctcaggtcgcagacgttttgcagcagcagtcgcttcacgttcgctcgcgtatcggtgattcattctgctaaccagtaaggcaaccccgccagcctagccgggtcctcaacgacaggagcacgatcatgcgcacccgtggccaggacccaacgctgcccgaaatt

SEQ ID NO: 21 - DNA, 35 bp, Artificial Sequence
  primer
aagcttggcactggccgtcgttttacaacgtcgtg

SEQ ID NO: 22 - DNA, 35 bp, Artificial Sequence
  primer
ggatccgaattctgaaatccttccctcgatcccga

SEQ ID NO: 23 - DNA, 1770 bp, Homo sapiens
aataaatgtagcagcgataaagcaattcagtttccgcgtcgtagcagcagcggttttcgtgttgatggttttgaaaaacgtgcagcagccagcgaaagcaataactatatgaatcatgttgccaaacagcagagcgaagaagcatttccgcaagaacagcagaaagcaccgcctgttgttggtggttttaatagcaatgttggtagcaaagttctgggcctgaaatatgaagaaattgactgcctgatcaacgatgagcataccattaaaggtcgtcgtgaaggtaatgaagtttttctgccgtttacctgggtggagaaatactttgatgtttatggtaaagtggtgcagtatgatggctatgatcgttttgaatttagccatagctacagcaaagtttatgcacagcgtgcaccgtatcatcctgatggtgtttttatgagctttgagggctataatgttgaagttcgtgatcgcgttaaatgcattagcggtgttgaaggtgttccgctgagcacccagtggggtccgcagggttatttctatccgattcagattgcacagtatggcctgagccattatagcaaaaatctgaccgaaaaaccgcctcacattgaagtttatgaaaccgcagaagatcgcgacaaaaacaaaccgaatgattggaccgttccgaaaggttgttttatggcaaatgttgcagataaaagccgcttcaccaatgtgaaacagtttattgcaccggaaaccagcgaaggtgttagcctgcagctgggtaataccaaagattttatcattagcttcgatctgaaatttctgaccaatggtagcgttagcgttgttctggaaaccaccgaaaaaaatcagctgtttaccatccattatgtgagcaatgcccagctgattgcatttaaagaacgcgatatctattatggcattggtccgcgtaccagttggagcaccgttacccgtgatctggttaccgatctgcgtaaaggtgttggtctgagcaatacaaaagcagttaaaccgaccaaaattatgccgaaaaaagttgttcgtctgatcgccaaaggtaaaggttttctggataacattaccattagcaccaccgcacatatggcagcattttttgcagcaagcgattggctggttcgtaaccaggatgaaaaaggtggttggccgattatggttacccgtaaactgggtgaaggttttaaaagcctggaaccgggttggtatagcgcaatggcacagggtcaggcaattagcaccctggttcgtgcatatctgctgaccaaagatcatatttttctgaatagcgcactgcgtgcaaccgcaccgtacaaatttctgtcagaacagcatggtgttaaagccgtgtttatgaacaaacacgattggtatgaagaatatccgaccaccccgagcagctttgttctgaatggttttatgtatagcctgatcggtctgtacgacctgaaagaaacagccggtgaaaaactgggtaaagaagcacgtagcctgtacgaacgtggtatggaaagcctgaaagcaatgctgccgctgtatgataccggtagcggcaccatttatgatctgcgtcattttatgctgggtatcgcaccgaatctggcacgttgggattatcataccacccatattaatcagctgcaactgctgagtaccattgatgaaagtccggtgtttaaagaatttgtgaaacgctggaaaagctacctgaaaggtagccgtgcaaaacacaattaa

SEQ ID NO: 24 - protein, 589 aa, Homo sapiens
NKCSSDKAIQFPRRSSSGFRVDGFEKRAAASESNNYMNHVAKQQSEEAFPQEQQKAPPVVGGFNSNVGSKVLGLKYEEIDCLINDEHTIKGRREGNEVFLPFTWVEKYFDVYGKVVQYDGYDRFEFSHSYSKVYAQRAPYHPDGVFMSFEGYNVEVRDRVKCISGVEGVPLSTQWGPQGYFYPIQIAQYGLSHYSKNLTEKPPHIEVYETAEDRDKNKPNDWTVPKGCFMANVADKSRFTNVKQFIAPETSEGVSLQLGNTKDFIISFDLKFLTNGSVSVVLETTEKNQLFTIHYVSNAQLIAFKERDIYYGIGPRTSWSTVTRDLVTDLRKGVGLSNTKAVKPTKIMPKKVVRLIAKGKGFLDNITISTTAHMAAFFAASDWLVRNQDEKGGWPIMVTRKLGEGFKSLEPGWYSAMAQGQAISTLVRAYLLTKDHIFLNSALRATAPYKFLSEQHGVKAVFMNKHDWYEEYPTTPSSFVLNGFMYSLIGLYDLKETAGEKLGKEARSLYERGMESLKAMLPLYDTGSGTIYDLRHFMLGIAPNLARWDYHTTHINQLQLLSTIDESPVFKEFVKRWKSYLKGSRAKHN

SEQ ID NO: 25 - DNA, 36 bp, Artificial Sequence
  primer
ttcagaattcggatcccgtgaaattgaacagcgtca

SEQ ID NO: 26 - DNA, 36 bp, Artificial Sequence
  primer
ggccagtgccaagcttttaattgcttttcggataga

SEQ ID NO: 27 - DNA, 918 bp, Cricetulus griseus
cgtgaaattgaacagcgtcataccatggatggtccgcgtcaggatgcagcagttgatgaagaagaagatatcgtcattatctataaccgtgttccgaaaaccgcaagcaccagctttaccaatattgcaattgatctgtgcgccaaaaatcgctatcatgtgctgcatatcaacaccaccaaaaataacccggttatgagcctgcaggatcaggttcgttttgttaaaaacattaccacctggaacgaaatgaaaccgggtttttatcatggccatatcagctatctggattttgcgaaatttggcgtgaaaaaaaaaccgatctacatcaacgttattcgcgatccgattgaacgtctggttagctattattactttctgcgcttcggtgatgattatcgtccgggtctgcgtcgtcgtaaacagggcgacaaaaaaacctttgatgaatgtgttgccgaaggtggtagcgattgtgcaccggaaaaactgtggctgcagattccgtttttttgcggtcatagcagcgaatgttggaatgttggtagccgttgggcaatggatcaggccaaatataacctgatcaacgaatattttctggtgggtgtgaccgaagaactggaagatttcattatgctgctggaagcagcactgcctcgtttttttcgtggtgcaaccgatctgtatcgtaccggtaaaaaaagccatctgcgtaaaacgacggaaaaaaaactgccgaccaaacagaccattgcaaaactgcagcagagcgatatttggaaaatggaaaacgagttttatgaatttgccctggaacagtttcagtttattcgtgcacatgcagttcgtgaaaaagatggtgatctgtatattctggcccagaacttcttctacgaaaaaatctatccgaaaagcaat

SEQ ID NO: 28 - protein, 306 aa, Cricetulus griseus
REIEQRHTMDGPRQDAAVDEEEDIVIIYNRVPKTASTSFTNIAIDLCAKNRYHVLHINTTKNNPVMSLQDQVRFVKNITTWNEMKPGFYHGHISYLDFAKFGVKKKPIYINVIRDPIERLVSYYYFLRFGDDYRPGLRRRKQGDKKTFDECVAEGGSDCAPEKLWLQIPFFCGHSSECWNVGSRWAMDQAKYNLINEYFLVGVTEELEDFIMLLEAALPRFFRGATDLYRTGKKSHLRKTTEKKLPTKQTIAKLQQSDIWKMENEFYEFALEQFQFIRAHAVREKDGDLYILAQNFFYEKIYPKSN

SEQ ID NO: 29 - protein, 311 aa, Mus musculus [sequence omitted]

SEQ ID NO: 30 - DNA, 808 bp, Artificial Sequence
  3-OST-1 gene optimized for expression of E. coli
gaattcgggcaccgcaagcaatggtagcacccagcagctgccgcagaccattattatcggtgttcgtaaaggtggcacccgtgcactgctggaaatgctgagcctgcatcctgatgttgcagcagcagaaaatgaagtgcatttttttgattgggaggaacattatagccagggtctgggttggtatctgacccagatgccgtttagcagtccgcatcagctgaccgttgaaaaaacaccggcatatttcaccagcccgaaagtgccggaacgtattcatagcatgaatccgaccattcgcctgctgctgattctgcgtgatccgagcgaacgtgttctgagcgattatacccaggttctgtataatcatctgcagaaacataaaccgtatccgcctattgaagatctgctgatgcgtgatggtcgtctgaatctggattataaagcactgaatcgtagcctgtatcatgcccatatgctgaattggctgcgtttttttccgctgggtcatattcatattgttgatggtgatcgtctgattcgtgatccgtttcctgaaattcagaaagtggaacgttttctgaaactgagtccgcagattaatgccagcaacttctattttaacaaaaccaaaggcttctattgcctgcgtgatagcggtaaagatcgttgtctgcatgaaagcaaaggtcgtgcacatccgcaggttgatccgaaactgctggataaactgcatgaatattttcatgaaccgaacaaaaaattctttaaactggtgggtcgtaccttcgattggcattaagtcgac

SEQ ID NO: 31 - DNA, 26 bp, Artificial Sequence
  primer
ataagatctgctgccgaacccgccaa

SEQ ID NO: 32 - DNA, 59 bp, Artificial Sequence
  primer
ataaagcttggatccgagctcgaggcggccgccagggctgcatcgacagtctgacgacc

SEQ ID NO: 33 - DNA, 6556 bp, Artificial Sequence
  plasmid
ccgacaccatcgaatggtgcaaaacctttcgcggtatggcatgatagcgcccggaagagagtcaattcagggtggtgaatgtgaaaccagtaacgttatacgatgtcgcagagtatgccggtgtctcttatcagaccgtttcccgcgtggtgaaccaggccagccacgtttctgcgaaaacgcgggaaaaagtggaagcggcgatggcggagctgaattacattcccaaccgcgtggcacaacaactggcgggcaaacagtcgttgctgattggcgttgccacctccagtctggccctgcacgcgccgtcgcaaattgtcgcggcgattaaatctcgcgccgatcaactgggtgccagcgtggtggtgtcgatggtagaacgaagcggcgtcgaagcctgtaaagcggcggtgcacaatcttctcgcgcaacgcgtcagtgggctgatcattaactatccgctggatgaccaggatgccattgctgtggaagctgcctgcactaatgttccggcgttatttcttgatgtctctgaccagacacccatcaacagtattattttctcccatgaagacggtacgcgactgggcgtggagcatctggtcgcattgggtcaccagcaaatcgcgctgttagcgggcccattaagttctgtctcggcgcgtctgcgtctggctggctggcataaatatctcactcgcaatcaaattcagccgatagcggaacgggaaggcgactggagtgccatgtccggttttcaacaaaccatgcaaatgctgaatgagggcatcgttcccactgcgatgctggttgccaacgatcagatggcgctgggcgcaatgcgcgccattaccgagtccgggctgcgcgttggtgcggatatctcggtagtgggatacgacgataccgaagacagctcatgttatatcccgccgttaaccaccatcaaacaggattttcgcctgctggggcaaaccagcgtggaccgcttgctgcaactctctcagggccaggcggtgaagggcaatcagctgttgcccgtctcactggtgaaaagaaaaaccaccctggcgcccaatacgcaaaccgcctctccccgcgcgttggccgattcattaatgcagctggcacgacaggtttcccgactggaaagcgggcagtgagcgcaacgcaattaatgtaagttagctcactcattaggcacaattctcatgtttgacagcttatcatcgactgcacggtgcaccaatgcttctggcgtcaggcagccatcggaagctgtggtatggctgtgcaggtcgtaaatcactgcataattcgtgtcgctcaaggcgcactcccgttctggataatgttttttgcgccgacatcataacggttctggcaaatattctgaaatgagctgttgacaattaatcatcggctcgtataatgtgtggaattgtgagcggataacaatttcacacaggaaacagccagtccgtttaggtgttttcacgagcacttcaccaacaaggaccatagcatatgaaaatcgaagaaggtaaactggtaatctggattaacggcgataaaggctataacggtctcgctgaagtcggtaagaaattcgagaaagataccggaattaaagtcaccgttgagcatccggataaactggaagagaaattcccacaggttgcggcaactggcgatggccctgacattatcttctgggcacacgaccgctttggtggctacgctcaatctggcctgttggctgaaatcaccccggacaaagcgttccaggacaagctgtatccgtttacctgggatgccgtacgttacaacggcaagctgattgcttacccgatcgctgttgaagcgttatcgctgatttataacaaagatctgctgccgaacccgccaaaaacctgggaagagatcccggcgctggataaagaactgaaagcgaaaggtaagagcgcgctgatgttcaacctgcaagaaccgtacttcacctggccgctgattgctgctgacgggggttatgcgttcaagtatgaaaacggcaagtacgacattaaagacgtgggcgtggataacgctggcgcgaaagcgggtctgaccttcctggttgacctgattaaaaacaaacacatgaatgcagacaccgattactccatcgcagaagctgcctttaataaaggcgaaacagcgatgaccatcaacggcccgtgggcatggtccaacatcgacaccagcaaagtgaattatggtgtaacggtactgccgaccttcaagggtcaaccatccaaaccgttcgttggcgtgctgagcgcaggtattaacgccgccagtccgaacaaagagctggcaaaagagttcctcgaaaactatctgctgactgatgaaggtctggaagcggttaataaagacaaaccgctgggtgccgtagcgctgaagtcttacgaggaagagttggcgaaagatccacgtattgccgccactatggaaaacgcccagaaaggtgaaatcatgccgaacatcccgcagatgtccgctttctggtatgccgtgcgtactgcggtgatcaacgccgccagcggtcgtcagactgtcgatgcagccctggcggccgcctcgagctcggatccaagcttggcactggccgtcgttttacaacgtcgtgactgggaaaaccctggcgttacccaacttaatcgccttgcagcacatccccctttcgccagctggcgtaatagcgaagaggcccgcaccgatcgcccttcccaacagttgcgcagcctgaatggcgaatggcagcttggctgttttggcggatgagataagattttcagcctgatacagattaaatcagaacgcagaagcggtctgataaaacagaatttgcctggcggcagtagcgcggtggtcccacctgaccccatgccgaactcagaagtgaaacgccgtagcgccgatggtagtgtggggtctccccatgcgagagtagggaactgccaggcatcaaataaaacgaaaggctcagtcgaaagactgggcctttcgttttatctgttgtttgtcggtgaacgctctcctgagtaggacaaatccgccgggagcggatttgaacgttgcgaagcaacggcccggagggtggcgggcaggacgcccgccataaactgccaggcatcaaattaagcagaaggccatcctgacggatggcctttttgcgtttctacaaactctttttgtttatttttctaaatacattcaaatatgtatccgctcatgagacaataaccctgataaatgcttcaataatattgaaaaaggaagagtatgagtattcaacatttccgtgtcgcccttattcccttttttgcggcattttgccttcctgtttttgctcacccagaaacgctggtgaaagtaaaagatgctgaagatcagttgggtgcacgagtgggttacatcgaactggatctcaacagcggtaagatccttgagagttttcgccccgaagaacgttctccaatgatgagcacttttaaagttctgctatgtggcgcggtattatcccgtgttgacgccgggcaagagcaactcggtcgccgcatacactattctcagaatgacttggttgagtactcaccagtcacagaaaagcatcttacggatggcatgacagtaagagaattatgcagtgctgccataaccatgagtgataacactgcggccaacttacttctgacaacgatcggaggaccgaaggagctaaccgcttttttgcacaacatgggggatcatgtaactcgccttgatcgttgggaaccggagctgaatgaagccataccaaacgacgagcgtgacaccacgatgcctgtagcaatggcaacaacgttgcgcaaactattaactggcgaactacttactctagcttcccggcaacaattaatagactggatggaggcggataaagttgcaggaccacttctgcgctcggcccttccggctggctggtttattgctgataaatctggagccggtgagcgtgggtctcgcggtatcattgcagcactggggccagatggtaagccctcccgtatcgtagttatctacacgacggggagtcaggcaactatggatgaacgaaatagacagatcgctgagataggtgcctcactgattaagcattggtaactgtcagaccaagtttactcatatatactttagattgatttaccccggttgataatcagaaaagccccaaaaacaggaagattgtataagcaaatatttaaattgtaaacgttaatattttgttaaaattcgcgttaaatttttgttaaatcagctcattttttaaccaataggccgaaatcggcaaaatcccttataaatcaaaagaatagaccgagatagggttgagtgttgttccagtttggaacaagagtccactattaaagaacgtggactccaacgtcaaagggcgaaaaaccgtctatcagggcgatggcccactacgtgaaccatcacccaaatcaagttttttggggtcgaggtgccgtaaagcactaaatcggaaccctaaagggagcccccgatttagagcttgacggggaaagccggcgaacgtggcgagaaaggaagggaagaaagcgaaaggagcgggcgctagggcgctggcaagtgtagcggtcacgctgcgcgtaaccaccacacccgccgcgcttaatgcgccgctacagggcgcgtaaaaggatctaggtgaagatcctttttgataatctcatgaccaaaatcccttaacgtgagttttcgttccactgagcgtcagaccccgtagaaaagatcaaaggatcttcttgagatcctttttttctgcgcgtaatctgctgcttgcaaacaaaaaaaccaccgctaccagcggtggtttgtttgccggatcaagagctaccaactctttttccgaaggtaactggcttcagcagagcgcagataccaaatactgtccttctagtgtagccgtagttaggccaccacttcaagaactctgtagcaccgcctacatacctcgctctgctaatcctgttaccagtggctgctgccagtggcgataagtcgtgtcttaccgggttggactcaagacgatagttaccggataaggcgcagcggtcgggctgaacggggggttcgtgcacacagcccagcttggagcgaacgacctacaccgaactgagatacctacagcgtgagctatgagaaagcgccacgcttcccgaagggagaaaggcggacaggtatccggtaagcggcagggtcggaacaggagagcgcacgagggagcttccagggggaaacgcctggtatctttatagtcctgtcgggtttcgccacctctgacttgagcgtcgatttttgtgatgctcgtcaggggggcggagcctatggaaaaacgccagcaacgcggcctttttacggttcctggccttttgctggccttttgctcacatgttctttcctgcgttatcccctgattctgtggataaccgtattaccgcctttgagtgagctgataccgctcgccgcagccgaacgaccgagcgcagcgagtcagtgagcgaggaagcggaagagcgcctgatgcggtattttctccttacgcatctgtgcggtatttcacaccgcatatatggtgcactctcagtacaatctgctctgatgccgcatagttaagccagtatacactccgctatcgctacgtgactgggtcatggctgcgccccgacacccgccaacacccgctgacgcgccctgacgggcttgtctgctcccggcatccgcttacagacaagctgtgaccgtctccgggagctgcatgtgtcagaggttttcaccgtcatcaccgaaacgcgcgaggcagctgcggtaaagctcatcagcgtggtcgtgcagcgattcacagatgtctgcctgttcatccgcgtccagctcgttgagtttctccagaagcgttaatgtctggcttctgataaagcgggccatgttaagggcggttttttcctgtttggtcactgatgcctccgtgtaagggggatttctgttcatgggggtaatgataccgatgaaacgagagaggatgctcacgatacgggttactgatgatgaacatgcccggttactggaacgttgtgagggtaaacaactggcggtatggatgcggcgggaccagagaaaaatcactcagggtcaatgccagcgcttcgttaatacagatgtaggtgttccacagggtagccagcagcatcctgcgatgcagatccggaacataatggtgcagggcgctgacttccgcgtttccagactttacgaaacacggaaaccgaagaccattcatgttgttgctcaggtcgcagacgttttgcagcagcagtcgcttcacgttcgctcgcgtatcggtgattcattctgctaaccagtaaggcaaccccgccagcctagccgggtcctcaacgacaggagcacgatcatgcgcacccgtggccaggacccaacgctgcccgaaatt

SEQ ID NO: 34 - DNA, 48 bp, Artificial Sequence
  primer
atagcggccgcgtcttctggaggcctgaaatatgaagaaattgactgc

SEQ ID NO: 35 - DNA, 31 bp, Artificial Sequence
  primer
atactcgagttaattgtgttttgcacggcta

SEQ ID NO: 36 - DNA, 1575 bp, Homo sapiens
ggccgcgtcttctggaggcctgaaatatgaagaaattgactgcctgatcaacgatgagcataccattaaaggtcgtcgtgaaggtaatgaagtttttctgccgtttacctgggtggagaaatactttgatgtttatggtaaagtggtgcagtatgatggctatgatcgttttgaatttagccatagctacagcaaagtttatgcacagcgtgcaccgtatcatcctgatggtgtttttatgagctttgagggctataatgttgaagttcgtgatcgcgttaaatgcattagcggtgttgaaggtgttccgctgagcacccagtggggtccgcagggttatttctatccgattcagattgcacagtatggcctgagccattatagcaaaaatctgaccgaaaaaccgcctcacattgaagtttatgaaaccgcagaagatcgcgacaaaaacaaaccgaatgattggaccgttccgaaaggttgttttatggcaaatgttgcagataaaagccgcttcaccaatgtgaaacagtttattgcaccggaaaccagcgaaggtgttagcctgcagctgggtaataccaaagattttatcattagcttcgatctgaaatttctgaccaatggtagcgttagcgttgttctggaaaccaccgaaaaaaatcagctgtttaccatccattatgtgagcaatgcccagctgattgcatttaaagaacgcgatatctattatggcattggtccgcgtaccagttggagcaccgttacccgtgatctggttaccgatctgcgtaaaggtgttggtctgagcaatacaaaagcagttaaaccgaccaaaattatgccgaaaaaagttgttcgtctgatcgccaaaggtaaaggttttctggataacattaccattagcaccaccgcacatatggcagcattttttgcagcaagcgattggctggttcgtaaccaggatgaaaaaggtggttggccgattatggttacccgtaaactgggtgaaggttttaaaagcctggaaccgggttggtatagcgcaatggcacagggtcaggcaattagcaccctggttcgtgcatatctgctgaccaaagatcatatttttctgaatagcgcactgcgtgcaaccgcaccgtacaaatttctgtcagaacagcatggtgttaaagccgtgtttatgaacaaacacgattggtatgaagaatatccgaccaccccgagcagctttgttctgaatggttttatgtatagcctgatcggtctgtacgacctgaaagaaacagccggtgaaaaactgggtaaagaagcacgtagcctgtacgaacgtggtatggaaagcctgaaagcaatgctgccgctgtatgataccggtagcggcaccatttatgatctgcgtcattttatgctgggtatcgcaccgaatctggcacgttgggattatcataccacccatattaatcagctgcaactgctgagtaccattgatgaaagtccggtgtttaaagaatttgtgaaacgctggaaaagctacctgaaaggtagccgtgcaaaacacaattaactcga

SEQ ID NO: 37 - protein, 517 aa, Homo sapiens
GLKYEEIDCLINDEHTIKGRREGNEVFLPFTWVEKYFDVYGKVVQYDGYDRFEFSHSYSKVYAQRAPYHPDGVFMSFEGYNVEVRDRVKCISGVEGVPLSTQWGPQGYFYPIQIAQYGLSHYSKNLTEKPPHIEVYETAEDRDKNKPNDWTVPKGCFMANVADKSRFTNVKQFIAPETSEGVSLQLGNTKDFIISFDLKFLTNGSVSVVLETTEKNQLFTIHYVSNAQLIAFKERDIYYGIGPRTSWSTVTRDLVTDLRKGVGLSNTKAVKPTKIMPKKVVRLIAKGKGFLDNITISTTAHMAAFFAASDWLVRNQDEKGGWPIMVTRKLGEGFKSLEPGWYSAMAQGQAISTLVRAYLLTKDHIFLNSALRATAPYKFLSEQHGVKAVFMNKHDWYEEYPTTPSSFVLNGFMYSLIGLYDLKETAGEKLGKEARSLYERGMESLKAMLPLYDTGSGTIYDLRHFMLGIAPNLARWDYHTTHINQLQLLSTIDESPVFKEFVKRWKSYLKGSRAKHN

SEQ ID NO: 38 - DNA, 63 bp, Artificial Sequence
  primer
atagcggccgcgcagactaatgcagcagcggatgaagaagaagatatcgtcattatctataac

SEQ ID NO: 39 - DNA, 36 bp, Artificial Sequence
  primer
atactcgagttaattgcttttcggatagattttttc

SEQ ID NO: 40 - DNA, 897 bp, Cricetulus griseus
ggccgcgcagactaatgcagcagcggatgaagaagaagatatcgtcattatctataaccgtgttccgaaaaccgcaagcaccagctttaccaatattgcatatgatctgtgcgccaaaaatcgctatcatgtgctgcatattaacaccaccaaaaataacccggttatgagcctgcaggatcaggttcgttttgttaaaaacattaccacctggaacgaaatgaaaccgggtttttatcatggccatatcagctatctggattttgcgaaatttggcgtgaaaaaaaaaccgatctacatcaacgttattcgcgatccgattgaacgtctggttagctattattactttctgcgcttcggtgatgattatcgtccgggtctgcgtcgtcgtaaacagggcgacaaaaaaacctttgatgaatgtgttgccgaaggtggtagcgattgtgcaccggaaaaactgtggctgcagattccgtttttttgcggtcatagcagcgaatgttggaatgttggtagccgttgggcaatggatcaggccaaatataacctgatcaacgaatattttctggtgggtgtgaccgaagaactggaagatttcattatgctgctggaagcagcactgcctcgtttttttcgtggtgcaaccgatctgtatcgtaccggtaaaaaaagccatctgcgtaaaacgacggaaaaaaaactgccgaccaaacagaccattgcaaaactgcagcagagcgatatttggaaaatggaaaacgagttttatgaatttgccctggaacagtttcagtttattcgtgcacatgcagttcgtgaaaaagatggtgatctgtatattctggcccagaacttcttctacgaaaaaatctatccgaaaagcaattaactcga

SEQ ID NO: 41 - protein, 288 aa, Cricetulus griseus
DEEEDIVIIYNRVPKTASTSFTNIAYDLCAKNRYHVLHINTTKNNPVMSLQDQVRFVKNITTWNEMKPGFYHGHISYLDFAKFGVKKKPIYINVIRDPIERLVSYYYFLRFGDDYRPGLRRRKQGDKKTFDECVAEGGSDCAPEKLWLQIPFFCGHSSECWNVGSRWAMDQAKYNLINEYFLVGVTEELEDFIMLLEAALPRFFRGATDLYRTGKKSHLRKTTEKKLPTKQTIAKLQQSDIWKMENEFYEFALEQFQFIRAHAVREKDGDLYILAQNFFYEKIYPKSN